European Patent Specification EP 4 251 200 B1, published October 30, 2024. Title: NOVEL REPLICATION DEFICIENT INFLUENZA A VIRUS INDUCING HIGH LEVELS OF TYPE I INTERFERON. Applicant: BlueSky Immunotherapies GmbH. The sequence listing filed with the application follows.

SEQUENCE LISTING (12 sequences)

SEQ ID NO: 1 - protein, 230 aa, Artificial Sequence
  Amino acid sequence of full length NS1 protein
MDPNTVSSFQVDCFLWHVRKRVADQELGDAPFLDRLRRDQKSLRGRGSTLGLDIETATRAGKQIVERILKEESDEALKMTMASVPASRYLTDMTLEEMSRDWSMLIPKQKVAGPLCIRMDQAIMDKNIILKANFSVIFDRLETLILLRAFTEEGAIVGEISPLPSLPGHTAEDVKNAVGVLIGGLEWNDNTVRVSETLQRFAWRSSNENGRPPLTPKQKREMAGTIRSEV

SEQ ID NO: 2 - DNA, 890 bp, Artificial Sequence
  Nucleotide sequence of full length NS gene
agcaaaagcagggtgacaaagacataatggatccaaacactgtgtcaagctttcaggtagattgctttctttggcatgtccgcaaacgagttgcagaccaagaactaggtgatgccccattccttgatcggcttcgccgagatcagaaatccctaagaggaaggggcagcaccctcggtctggacatcgagacagccacacgtgctggaaagcagatagtggagcggattctgaaagaagaatccgatgaggcacttaaaatgaccatggcctctgtacctgcgtcgcgttacctaactgacatgactcttgaggaaatgtcaagggactggtccatgctcatacccaagcagaaagtggcaggccctctttgtatcagaatggaccaggcgatcatggataagaacatcatactgaaagcgaacttcagtgtgatttttgaccggctggagactctaatattgctaagggctttcaccgaagagggagcaattgttggcgaaatttcaccattgccttctcttccaggacatactgctgaggatgtcaaaaatgcagttggagtcctcatcgggggacttgaatggaatgataacacagttcgagtctctgaaactctacagagattcgcttggagaagcagtaatgagaatgggagacctccactcactccaaaacagaaacgagaaatggcgggaacaattaggtcagaagtttgaagaaataagatggttgattgaagaagtgagacacaaactgaagataacagagaatagttttgagcaaataacatttatgcaagccttacatctattgcttgaagtggagcaagagataagaactttctcgtttcagcttatttaataataaaaaacacccttgtttctact

SEQ ID NO: 3 - protein, 171 aa, Artificial Sequence
  Amino acid sequence DelNS15-73
MDPNTVSSFQVDCFDEALKMTMASVPASRYLTDMTLEEMSRDWSMLIPKQKVAGPLCIRMDQAIMDKNIILKANFSVIFDRLETLILLRAFTEEGAIVGEISPLPSLPGHTAEDVKNAVGVLIGGLEWNDNTVRVSETLQRFAWRSSNENGRPPLTPKQKREMAGTIRSEV

SEQ ID NO: 4 - DNA, 713 bp, Artificial Sequence
  Nt sequence DelNS15-73
agcaaaagcagggtgacaaagacataatggatccaaacactgtgtcaagctttcaggtagattgctttgatgaggcacttaaaatgaccatggcctctgtacctgcgtcgcgttacctaactgacatgactcttgaggaaatgtcaagggactggtccatgctcatacccaagcagaaagtggcaggccctctttgtatcagaatggaccaggcgatcatggataagaacatcatactgaaagcgaacttcagtgtgatttttgaccggctggagactctaatattgctaagggctttcaccgaagagggagcaattgttggcgaaatttcaccattgccttctcttccaggacatactgctgaggatgtcaaaaatgcagttggagtcctcatcgggggacttgaatggaatgataacacagttcgagtctctgaaactctacagagattcgcttggagaagcagtaatgagaatgggagacctccactcactccaaaacagaaacgagaaatggcgggaacaattaggtcagaagtttgaagaaataagatggttgattgaagaagtgagacacaaactgaagataacagagaatagttttgagcaaataacatttatgcaagccttacatctattgcttgaagtggagcaagagataagaactttctcgtttcagcttatttaataataaaaaacacccttgtttctact

SEQ ID NO: 5 - protein, 214 aa, Artificial Sequence
  Amino acid sequence of DelNS35-50
MDPNTVSSFQVDCFLWHVRKRVADQELGDAPFLDGLDIETATRAGKQIVERILKEESDEALKMTMASVPASRYLTDMTLEEMSRDWSMLIPKQKVAGPLCIRMDQAIMDKNIILKANFSVIFDRLETLILLRAFTEEGAIVGEISPLPSLPGHTAEDVKNAVGVLIGGLEWNDNTVRVSETLQRFAWRSSNENGRPPLTPKQKREMAGTIRSEV

SEQ ID NO: 6 - DNA, 842 bp, Artificial Sequence
  Nt sequence of DelNS35-50
agcaaaagcagggtgacaaagacataatggatccaaacactgtgtcaagctttcaggtagattgctttctttggcatgtccgcaaacgagttgcagaccaagaactaggtgatgccccattccttgatggtctggacatcgagacagccacacgtgctggaaagcagatagtggagcggattctgaaagaagaatccgatgaggcacttaaaatgaccatggcctctgtacctgcgtcgcgttacctaactgacatgactcttgaggaaatgtcaagggactggtccatgctcatacccaagcagaaagtggcaggccctctttgtatcagaatggaccaggcgatcatggataagaacatcatactgaaagcgaacttcagtgtgatttttgaccggctggagactctaatattgctaagggctttcaccgaagagggagcaattgttggcgaaatttcaccattgccttctcttccaggacatactgctgaggatgtcaaaaatgcagttggagtcctcatcgggggacttgaatggaatgataacacagttcgagtctctgaaactctacagagattcgcttggagaagcagtaatgagaatgggagacctccactcactccaaaacagaaacgagaaatggcgggaacaattaggtcagaagtttgaagaaataagatggttgattgaagaagtgagacacaaactgaagataacagagaatagttttgagcaaataacatttatgcaagccttacatctattgcttgaagtggagcaagagataagaactttctcgtttcagcttatttaataataaaaaacacccttgtttctact

SEQ ID NO: 7 - protein, 194 aa, Artificial Sequence
  Amino acid sequence of DelNS35-70
MDPNTVSSFQVDCFLWHVRKRVADQELGDAPFLDEESDEALKMTMASVPASRYLTDMTLEEMSRDWSMLIPKQKVAGPLCIRMDQAIMDKNIILKANFSVIFDRLETLILLRAFTEEGAIVGEISPLPSLPGHTAEDVKNAVGVLIGGLEWNDNTVRVSETLQRFAWRSSNENGRPPLTPKQKREMAGTIRSEV

SEQ ID NO: 8 - DNA, 782 bp, Artificial Sequence
  Nt sequence of DelNS35-70
agcaaaagcagggtgacaaagacataatggatccaaacactgtgtcaagctttcaggtagattgctttctttggcatgtccgcaaacgagttgcagaccaagaactaggtgatgccccattccttgatgaagaatccgatgaggcacttaaaatgaccatggcctctgtacctgcgtcgcgttacctaactgacatgactcttgaggaaatgtcaagggactggtccatgctcatacccaagcagaaagtggcaggccctctttgtatcagaatggaccaggcgatcatggataagaacatcatactgaaagcgaacttcagtgtgatttttgaccggctggagactctaatattgctaagggctttcaccgaagagggagcaattgttggcgaaatttcaccattgccttctcttccaggacatactgctgaggatgtcaaaaatgcagttggagtcctcatcgggggacttgaatggaatgataacacagttcgagtctctgaaactctacagagattcgcttggagaagcagtaatgagaatgggagacctccactcactccaaaacagaaacgagaaatggcgggaacaattaggtcagaagtttgaagaaataagatggttgattgaagaagtgagacacaaactgaagataacagagaatagttttgagcaaataacatttatgcaagccttacatctattgcttgaagtggagcaagagataagaactttctcgtttcagcttatttaataataaaaaacacccttgtttctact

SEQ ID NO: 9 - protein, 209 aa, Artificial Sequence
  Amino acid sequence of DelNS40-60
MDPNTVSSFQVDCFLWHVRKRVADQELGDAPFLDRLRRDGKQIVERILKEESDEALKMTMASVPASRYLTDMTLEEMSRDWSMLIPKQKVAGPLCIRMDQAIMDKNIILKANFSVIFDRLETLILLRAFTEEGAIVGEISPLPSLPGHTAEDVKNAVGVLIGGLEWNDNTVRVSETLQRFAWRSSNENGRPPLTPKQKREMAGTIRSEV

SEQ ID NO: 10 - DNA, 827 bp, Artificial Sequence
  Nt sequence of DelNS40-60
agcaaaagcagggtgacaaagacataatggatccaaacactgtgtcaagctttcaggtagattgctttctttggcatgtccgcaaacgagttgcagaccaagaactaggtgatgccccattccttgatcggcttcgccgagatggaaagcagatagtggagcggattctgaaagaagaatccgatgaggcacttaaaatgaccatggcctctgtacctgcgtcgcgttacctaactgacatgactcttgaggaaatgtcaagggactggtccatgctcatacccaagcagaaagtggcaggccctctttgtatcagaatggaccaggcgatcatggataagaacatcatactgaaagcgaacttcagtgtgatttttgaccggctggagactctaatattgctaagggctttcaccgaagagggagcaattgttggcgaaatttcaccattgccttctcttccaggacatactgctgaggatgtcaaaaatgcagttggagtcctcatcgggggacttgaatggaatgataacacagttcgagtctctgaaactctacagagattcgcttggagaagcagtaatgagaatgggagacctccactcactccaaaacagaaacgagaaatggcgggaacaattaggtcagaagtttgaagaaataagatggttgattgaagaagtgagacacaaactgaagataacagagaatagttttgagcaaataacatttatgcaagccttacatctattgcttgaagtggagcaagagataagaactttctcgtttcagcttatttaataataaaaaacacccttgtttctact

SEQ ID NO: 11 - protein, 189 aa, Artificial Sequence
  Amino acid sequence of DelNS40-80
MDPNTVSSFQVDCFLWHVRKRVADQELGDAPFLDRLRRDMASVPASRYLTDMTLEEMSRDWSMLIPKQKVAGPLCIRMDQAIMDKNIILKANFSVIFDRLETLILLRAFTEEGAIVGEISPLPSLPGHTAEDVKNAVGVLIGGLEWNDNTVRVSETLQRFAWRSSNENGRPPLTPKQKREMAGTIRSEV

SEQ ID NO: 12 - DNA, 767 bp, Artificial Sequence
  Nt sequence of DelNS40-80
agcaaaagcagggtgacaaagacataatggatccaaacactgtgtcaagctttcaggtagattgctttctttggcatgtccgcaaacgagttgcagaccaagaactaggtgatgccccattccttgatcggcttcgccgagatatggcctctgtacctgcgtcgcgttacctaactgacatgactcttgaggaaatgtcaagggactggtccatgctcatacccaagcagaaagtggcaggccctctttgtatcagaatggaccaggcgatcatggataagaacatcatactgaaagcgaacttcagtgtgatttttgaccggctggagactctaatattgctaagggctttcaccgaagagggagcaattgttggcgaaatttcaccattgccttctcttccaggacatactgctgaggatgtcaaaaatgcagttggagtcctcatcgggggacttgaatggaatgataacacagttcgagtctctgaaactctacagagattcgcttggagaagcagtaatgagaatgggagacctccactcactccaaaacagaaacgagaaatggcgggaacaattaggtcagaagtttgaagaaataagatggttgattgaagaagtgagacacaaactgaagataacagagaatagttttgagcaaataacatttatgcaagccttacatctattgcttgaagtggagcaagagataagaactttctcgtttcagcttatttaataataaaaaacacccttgtttctact